European Patent Specification EP 3 825 413 B1, published March 6, 2024. Title: METHODS FOR IMPROVED ISOLATION OF GENOMIC DNA TEMPLATES FOR ALLELE DETECTION. Applicant: Avellino Lab USA, Inc. The sequence listing filed with the application follows.

SEQUENCE LISTING (42 sequences)

SEQ ID NO: 1 - DNA, 20 bp, Artificial
  primer
tccaccaccactcagctgta

SEQ ID NO: 2 - DNA, 19 bp, Artificial
  primer
ccatctcaggcctcagctt

SEQ ID NO: 3 - DNA, 20 bp, Artificial
  primer
tgcagccctaccactctcaa

SEQ ID NO: 4 - DNA, 16 bp, Artificial
  primer
aggcctcgttgctagg

SEQ ID NO: 5 - DNA, 20 bp, Artificial
  primer
tagtctcttattctaataga

SEQ ID NO: 6 - DNA, 20 bp, Artificial
  primer
gctgcagactctgtgtttaa

SEQ ID NO: 7 - DNA, 22 bp, Artificial
  primer
ccatccctccttctgtcttctg

SEQ ID NO: 8 - DNA, 16 bp, Artificial
  primer
cgggcccctccatctc

SEQ ID NO: 9 - DNA, 21 bp, Artificial
  primer
cagagaagggagggtgtggtt

SEQ ID NO: 10 - DNA, 19 bp, Artificial
  primer
gggcgaagatggtgaagct

SEQ ID NO: 11 - DNA, 21 bp, Artificial
  primer
tcctcgtcctctccacctgta

SEQ ID NO: 12 - DNA, 17 bp, Artificial
  primer
agctggcaaggaggccc

SEQ ID NO: 13 - DNA, 19 bp, Artificial
  primer
tttgggctttcccacatgc

SEQ ID NO: 14 - DNA, 20 bp, Artificial
  primer
ggcagacggaggtcatctca

SEQ ID NO: 15 - DNA, 18 bp, Artificial
  primer
gtagtaccgtgctctctg

SEQ ID NO: 16 - DNA, 21 bp, Artificial
  primer
agttccccataagaatccccc

SEQ ID NO: 17 - DNA, 17 bp, Artificial
  primer
ggctggacccccagagg

SEQ ID NO: 18 - DNA, 19 bp, Artificial
  primer
acccctcggggaagtaagg

SEQ ID NO: 19 - DNA, 21 bp, Artificial
  primer
aacctttacgagaccctggga

SEQ ID NO: 20 - DNA, 20 bp, Artificial
  primer
gactcccatccatcatgccc

SEQ ID NO: 21 - DNA, 20 bp, Artificial
  primer
agtcgttggatccaccacca

SEQ ID NO: 22 - DNA, 24 bp, Artificial
  primer
gacgtcatttcctactgtttcagg

SEQ ID NO: 23 - DNA, 18 bp, Artificial
  primer
ccccccagaaacagcctg

SEQ ID NO: 24 - DNA, 25 bp, Artificial
  primer
ttctaaggggttaaggagaaagctt

SEQ ID NO: 25 - DNA, 15 bp, Artificial
  probe
cacggaccgcacgga

SEQ ID NO: 26 - DNA, 15 bp, Artificial
  probe
cacggaccacacgga

SEQ ID NO: 27 - DNA, 14 bp, Artificial
  probe
acacggaccgcacg

SEQ ID NO: 28 - DNA, 14 bp, Artificial
  probe
acacggaccacacg

SEQ ID NO: 29 - DNA, 13 bp, Artificial
  probe
tacacggaccgca

SEQ ID NO: 30 - DNA, 13 bp, Artificial
  probe
tacacggaccaca

SEQ ID NO: 31 - DNA, 18 bp, Artificial
  probe
ctgtacacggaccgcacg

SEQ ID NO: 32 - DNA, 18 bp, Artificial
  probe
ctgtacacggaccacacg

SEQ ID NO: 33 - DNA, 21 bp, Artificial
  probe
ctgtacacggaccgcacggag

SEQ ID NO: 34 - DNA, 21 bp, Artificial
  probe
ctgtacacggaccacacggag

SEQ ID NO: 35 - DNA, 24 bp, Artificial
  probe
gctgtacacggaccgcacggagaa

SEQ ID NO: 36 - DNA, 24 bp, Artificial
  probe
gctgtacacggaccacacggagaa

SEQ ID NO: 37 - DNA, 15 bp, Artificial
  probe
accgcacggagaagc

SEQ ID NO: 38 - DNA, 15 bp, Artificial
  probe
accacacggagaagc

SEQ ID NO: 39 - DNA, 21 bp, Artificial
  probe
accgcacggagaagctgaggc

SEQ ID NO: 40 - DNA, 21 bp, Artificial
  probe
accacacggagaagctgaggc

SEQ ID NO: 41 - DNA, 24 bp, Artificial
  probe
accgcacggagaagctgaggcctg

SEQ ID NO: 42 - DNA, 24 bp, Artificial
  probe
accacacggagaagctgaggcctg